European Patent Application EP 4 335 924 A1, published March 13, 2024. Title: ULTRAPURE MINIVECTORS FOR GENE THERAPY. Applicant: BAYLOR COLLEGE OF MEDICINE & TWISTER BIOTECH, INC. Application US US 17/930,652, filed September 8, 2002. The sequence listing filed with the application follows.

SEQUENCE LISTING (162 sequences)

SEQ ID NO: 1 - DNA, 19 bp, synthetic construct
  misc_feature 1..19: note = Synthetic: V2LHS_237948
  source 1..19: mol_type = other DNA
aaattcatcatcgaagtac

SEQ ID NO: 2 - DNA, 19 bp, synthetic construct
  misc_feature 1..19: note = Synthetic: V2LHS_132502
  source 1..19: mol_type = other DNA
tgacaaaggtgttgggtcg

SEQ ID NO: 3 - DNA, 19 bp, synthetic construct
  misc_feature 1..19: note = Synthetic: V3LHS_636396
  source 1..19: mol_type = other DNA
gtgtgagcgacttcatcct

SEQ ID NO: 4 - DNA, 19 bp, synthetic construct
  misc_feature 1..19: note = Synthetic: V3LHS_646518
  source 1..19: mol_type = other DNA
tgatgctgaggaagaacct

SEQ ID NO: 5 - DNA, 19 bp, synthetic construct
  misc_feature 1..19: note = Synthetic: V3LHS_636398
  source 1..19: mol_type = other DNA
catcatcgaagtaccttgt

SEQ ID NO: 6 - DNA, 19 bp, synthetic construct
  misc_feature 1..19: note = Synthetic: V3LHS_636400
  source 1..19: mol_type = other DNA
ttgatgacagacacctcat

SEQ ID NO: 7 - DNA, 19 bp, synthetic construct
  misc_feature 1..19: note = Synthetic: V3LHS_325557
  source 1..19: mol_type = other DNA
tctttgatgacagacacct

SEQ ID NO: 8 - DNA, 19 bp, synthetic construct
  misc_feature 1..19: note = Synthetic: V2LHS_112035
  source 1..19: mol_type = other DNA
ttattaaagatgccacgtg

SEQ ID NO: 9 - DNA, 19 bp, synthetic construct
  misc_feature 1..19: note = Synthetic: V2LHS_265598
  source 1..19: mol_type = other DNA
aaagacaggaaatttcttg

SEQ ID NO: 10 - DNA, 19 bp, synthetic construct
  misc_feature 1..19: note = Synthetic: V2LHS_112039
  source 1..19: mol_type = other DNA
atgtctttggtaaacactc

SEQ ID NO: 11 - DNA, 19 bp, synthetic construct
  misc_feature 1..19: note = Synthetic: V2LHS_112037
  source 1..19: mol_type = other DNA
atccatgtgagaagaaatg

SEQ ID NO: 12 - DNA, 19 bp, synthetic construct
  misc_feature 1..19: note = Synthetic: V3LHS_398453
  source 1..19: mol_type = other DNA
actttgtctatatccatgt

SEQ ID NO: 13 - DNA, 19 bp, synthetic construct
  misc_feature 1..19: note = Synthetic: V3LHS_398455
  source 1..19: mol_type = other DNA
aattcaacagcattgtcca

SEQ ID NO: 14 - DNA, 19 bp, synthetic construct
  misc_feature 1..19: note = Synthetic: V2LHS_28602
  source 1..19: mol_type = other DNA
taagggaacagttagggat

SEQ ID NO: 15 - DNA, 19 bp, synthetic construct
  misc_feature 1..19: note = Synthetic: V2LHS_28606
  source 1..19: mol_type = other DNA
atgacagggaccatcaggc

SEQ ID NO: 16 - DNA, 19 bp, synthetic construct
  misc_feature 1..19: note = Synthetic: V2LHS_28601
  source 1..19: mol_type = other DNA
ttctccatcaccttctggc

SEQ ID NO: 17 - DNA, 19 bp, synthetic construct
  misc_feature 1..19: note = Synthetic: V3LHS_341839
  source 1..19: mol_type = other DNA
tcaagtagatcctcctccg

SEQ ID NO: 18 - DNA, 19 bp, synthetic construct
  misc_feature 1..19: note = Synthetic: V3LHS_341836
  source 1..19: mol_type = other DNA
atgtctctgtgaatcacct

SEQ ID NO: 19 - DNA, 19 bp, synthetic construct
  misc_feature 1..19: note = Synthetic: V3LHS_341841
  source 1..19: mol_type = other DNA
tcgatctctctgcgcagct

SEQ ID NO: 20 - DNA, 19 bp, synthetic construct
  misc_feature 1..19: note = Synthetic: V3LHS_341840
  source 1..19: mol_type = other DNA
agagcatctgccaactcct

SEQ ID NO: 21 - DNA, 19 bp, synthetic construct
  misc_feature 1..19: note = Synthetic: V3LHS_341837
  source 1..19: mol_type = other DNA
tttctggctttatgtctct

SEQ ID NO: 22 - DNA, 19 bp, synthetic construct
  misc_feature 1..19: note = Synthetic: V2LHS_62437
  source 1..19: mol_type = other DNA
ataatggtcgtgggttccc

SEQ ID NO: 23 - DNA, 19 bp, synthetic construct
  misc_feature 1..19: note = Synthetic: V2LHS_62435
  source 1..19: mol_type = other DNA
ttgcaaacacgttgagccg

SEQ ID NO: 24 - DNA, 19 bp, synthetic construct
  misc_feature 1..19: note = Synthetic: V3LHS_323253
  source 1..19: mol_type = other DNA
aatcctccactctgcagcc

SEQ ID NO: 25 - DNA, 19 bp, synthetic construct
  misc_feature 1..19: note = Synthetic: V3LHS_323254
  source 1..19: mol_type = other DNA
tccgctgtctttagctctg

SEQ ID NO: 26 - DNA, 19 bp, synthetic construct
  misc_feature 1..19: note = Synthetic: V3LHS_323256
  source 1..19: mol_type = other DNA
tgagtgtgacttcgtctcc

SEQ ID NO: 27 - DNA, 19 bp, synthetic construct
  misc_feature 1..19: note = Synthetic: V3LHS_323255
  source 1..19: mol_type = other DNA
gtgacttcgtctccttccc

SEQ ID NO: 28 - DNA, 19 bp, synthetic construct
  misc_feature 1..19: note = Synthetic: V3LHS_323251
  source 1..19: mol_type = other DNA
agaggtaaggaaagcacct

SEQ ID NO: 29 - DNA, 19 bp, synthetic construct
  misc_feature 1..19: note = Synthetic: V2LHS_94585
  source 1..19: mol_type = other DNA
atcaaatccatcatcttac

SEQ ID NO: 30 - DNA, 19 bp, synthetic construct
  misc_feature 1..19: note = Synthetic: V2LHS_94582
  source 1..19: mol_type = other DNA
taaacagtagaggagccag

SEQ ID NO: 31 - DNA, 19 bp, synthetic construct
  misc_feature 1..19: note = Synthetic: V2LHS_262796
  source 1..19: mol_type = other DNA
agcagaagaaacactgggc

SEQ ID NO: 32 - DNA, 19 bp, synthetic construct
  misc_feature 1..19: note = Synthetic: V2LHS_262484
  source 1..19: mol_type = other DNA
ttcctaagacattgctaag

SEQ ID NO: 33 - DNA, 19 bp, synthetic construct
  misc_feature 1..19: note = Synthetic: V2LHS_230582
  source 1..19: mol_type = other DNA
tcttgaatgtagagatgcg

SEQ ID NO: 34 - DNA, 19 bp, synthetic construct
  misc_feature 1..19: note = Synthetic: V3LHS_350788
  source 1..19: mol_type = other DNA
aattcttcaaactgcttct

SEQ ID NO: 35 - DNA, 19 bp, synthetic construct
  misc_feature 1..19: note = Synthetic: V3LHS_350789
  source 1..19: mol_type = other DNA
tgttcttggctctttctct

SEQ ID NO: 36 - DNA, 19 bp, synthetic construct
  misc_feature 1..19: note = Synthetic: V3LHS_383705
  source 1..19: mol_type = other DNA
tgaagcagaagaaacactg

SEQ ID NO: 37 - DNA, 19 bp, synthetic construct
  misc_feature 1..19: note = Synthetic: V3LHS_383704
  source 1..19: mol_type = other DNA
gaagcagaagaaacactgg

SEQ ID NO: 38 - DNA, 19 bp, synthetic construct
  misc_feature 1..19: note = Synthetic: V3LHS_369356
  source 1..19: mol_type = other DNA
ttaccatgactacattctt

SEQ ID NO: 39 - DNA, 19 bp, synthetic construct
  misc_feature 1..19: note = Synthetic: V3LHS_369358
  source 1..19: mol_type = other DNA
tgcttgcaataaacatggc

SEQ ID NO: 40 - DNA, 19 bp, synthetic construct
  misc_feature 1..19: note = Synthetic: V3LHS_369355
  source 1..19: mol_type = other DNA
taattttcgagttcctggt

SEQ ID NO: 41 - DNA, 19 bp, synthetic construct
  misc_feature 1..19: note = Synthetic: V3LHS_369360
  source 1..19: mol_type = other DNA
aaagctcttagaatcttca

SEQ ID NO: 42 - DNA, 19 bp, synthetic construct
  misc_feature 1..19: note = Synthetic: V3LHS_369359
  source 1..19: mol_type = other DNA
agaatcttcatttccatct

SEQ ID NO: 43 - DNA, 19 bp, synthetic construct
  misc_feature 1..19: note = Synthetic: V2LHS_71816
  source 1..19: mol_type = other DNA
atcattaagggattgatag

SEQ ID NO: 44 - DNA, 19 bp, synthetic construct
  misc_feature 1..19: note = Synthetic: V2LHS_71820
  source 1..19: mol_type = other DNA
ttatacaaatcaccaacag

SEQ ID NO: 45 - DNA, 19 bp, synthetic construct
  misc_feature 1..19: note = Synthetic: V2LHS_71818
  source 1..19: mol_type = other DNA
tagtagacaatctttagac

SEQ ID NO: 46 - DNA, 19 bp, synthetic construct
  misc_feature 1..19: note = Synthetic: V2LHS_71819
  source 1..19: mol_type = other DNA
tgttctataggaaggactc

SEQ ID NO: 47 - DNA, 19 bp, synthetic construct
  misc_feature 1..19: note = Synthetic: V3LHS_407402
  source 1..19: mol_type = other DNA
ttcattttagaacacttga

SEQ ID NO: 48 - DNA, 19 bp, synthetic construct
  misc_feature 1..19: note = Synthetic: V3LHS_352745
  source 1..19: mol_type = other DNA
ataggaaggactcgttgct

SEQ ID NO: 49 - DNA, 19 bp, synthetic construct
  misc_feature 1..19: note = Synthetic: V3LHS_352742
  source 1..19: mol_type = other DNA
atagtttcaacatcatcgt

SEQ ID NO: 50 - DNA, 19 bp, synthetic construct
  misc_feature 1..19: note = Synthetic: V3LHS_352743
  source 1..19: mol_type = other DNA
attattatacaaatcacca

SEQ ID NO: 51 - DNA, 19 bp, synthetic construct
  misc_feature 1..19: note = Synthetic: V2LHS_111680
  source 1..19: mol_type = other DNA
tatattcaaatcgatctgc

SEQ ID NO: 52 - DNA, 19 bp, synthetic construct
  misc_feature 1..19: note = Synthetic: V2LHS_111682
  source 1..19: mol_type = other DNA
atatgtgtcatactgggag

SEQ ID NO: 53 - DNA, 19 bp, synthetic construct
  misc_feature 1..19: note = Synthetic: V2LHS_111684
  source 1..19: mol_type = other DNA
aatggtgtaggtgttacac

SEQ ID NO: 54 - DNA, 19 bp, synthetic construct
  misc_feature 1..19: note = Synthetic: V3LHS_334831
  source 1..19: mol_type = other DNA
agagttggaatctccaaca

SEQ ID NO: 55 - DNA, 19 bp, synthetic construct
  misc_feature 1..19: note = Synthetic: V3LHS_334830
  source 1..19: mol_type = other DNA
tgggtctcttcttccacct

SEQ ID NO: 56 - DNA, 19 bp, synthetic construct
  misc_feature 1..19: note = Synthetic: V3LHS_334834
  source 1..19: mol_type = other DNA
tgtgcttgtagaatgtggg

SEQ ID NO: 57 - DNA, 19 bp, synthetic construct
  misc_feature 1..19: note = Synthetic: V3LHS_334832
  source 1..19: mol_type = other DNA
tgtctgaagtagcacttcc

SEQ ID NO: 58 - DNA, 19 bp, synthetic construct
  misc_feature 1..19: note = Synthetic: V2LHS_112883
  source 1..19: mol_type = other DNA
ttccagatgcgaatgtgtc

SEQ ID NO: 59 - DNA, 19 bp, synthetic construct
  misc_feature 1..19: note = Synthetic: V2LHS_112884
  source 1..19: mol_type = other DNA
ataactagctggttctgtg

SEQ ID NO: 60 - DNA, 19 bp, synthetic construct
  misc_feature 1..19: note = Synthetic: V3LHS_640507
  source 1..19: mol_type = other DNA
aactagctggttctgtgca

SEQ ID NO: 61 - DNA, 19 bp, synthetic construct
  misc_feature 1..19: note = Synthetic: V3LHS_640508
  source 1..19: mol_type = other DNA
caggtaatagtcatttcgg

SEQ ID NO: 62 - DNA, 19 bp, synthetic construct
  misc_feature 1..19: note = Synthetic: V3LHS_645717
  source 1..19: mol_type = other DNA
aaacaactgaggtgatggg

SEQ ID NO: 63 - DNA, 19 bp, synthetic construct
  misc_feature 1..19: note = Synthetic: V3LHS_645716
  source 1..19: mol_type = other DNA
aataaaaaacaactgaggt

SEQ ID NO: 64 - DNA, 19 bp, synthetic construct
  misc_feature 1..19: note = Synthetic: V3LHS_640514
  source 1..19: mol_type = other DNA
acttccaaataactagctg

SEQ ID NO: 65 - DNA, 19 bp, synthetic construct
  misc_feature 1..19: note = Synthetic: V3LHS_363298
  source 1..19: mol_type = other DNA
tctgctgctgcacatccca

SEQ ID NO: 66 - DNA, 19 bp, synthetic construct
  misc_feature 1..19: note = Synthetic: V2LHS_262156
  source 1..19: mol_type = other DNA
aataaatagaatccatttc

SEQ ID NO: 67 - DNA, 19 bp, synthetic construct
  misc_feature 1..19: note = Synthetic: V3LHS_401207
  source 1..19: mol_type = other DNA
atgaataactcataactca

SEQ ID NO: 68 - DNA, 19 bp, synthetic construct
  misc_feature 1..19: note = Synthetic: V3LHS_310385
  source 1..19: mol_type = other DNA
ccactaggaccttcagggt

SEQ ID NO: 69 - DNA, 19 bp, synthetic construct
  misc_feature 1..19: note = Synthetic: V3LHS_310386
  source 1..19: mol_type = other DNA
cgggatgcaccagctcgcg

SEQ ID NO: 70 - DNA, 19 bp, synthetic construct
  misc_feature 1..19: note = Synthetic: V3LHS_310389
  source 1..19: mol_type = other DNA
aggaccttcagggtgtcca

SEQ ID NO: 71 - DNA, 19 bp, synthetic construct
  misc_feature 1..19: note = Synthetic: V3LHS_310387
  source 1..19: mol_type = other DNA
gaactgccagatggattgg

SEQ ID NO: 72 - DNA, 19 bp, synthetic construct
  misc_feature 1..19: note = Synthetic: V2LHS_262397
  source 1..19: mol_type = other DNA
tatagtaggagacaagcag

SEQ ID NO: 73 - DNA, 19 bp, synthetic construct
  misc_feature 1..19: note = Synthetic: V2LHS_201585
  source 1..19: mol_type = other DNA
tgcttgatggtctgtattg

SEQ ID NO: 74 - DNA, 19 bp, synthetic construct
  misc_feature 1..19: note = Synthetic: V3LHS_386043
  source 1..19: mol_type = other DNA
tgattgtgaatctcttgat

SEQ ID NO: 75 - DNA, 19 bp, synthetic construct
  misc_feature 1..19: note = Synthetic: V3LHS_386040
  source 1..19: mol_type = other DNA
atcttgatacagatcttga

SEQ ID NO: 76 - DNA, 19 bp, synthetic construct
  misc_feature 1..19: note = Synthetic: V3LHS_386041
  source 1..19: mol_type = other DNA
tgatacagatcttgattgt

SEQ ID NO: 77 - DNA, 19 bp, synthetic construct
  misc_feature 1..19: note = Synthetic: V2LHS_150535
  source 1..19: mol_type = other DNA
atatgatggaaatgcccag

SEQ ID NO: 78 - DNA, 19 bp, synthetic construct
  misc_feature 1..19: note = Synthetic: V2LHS_150534
  source 1..19: mol_type = other DNA
tattacctctgttacagag

SEQ ID NO: 79 - DNA, 19 bp, synthetic construct
  misc_feature 1..19: note = Synthetic: V2LHS_150531
  source 1..19: mol_type = other DNA
taacacatatttctcttgc

SEQ ID NO: 80 - DNA, 19 bp, synthetic construct
  misc_feature 1..19: note = Synthetic: V3LHS_403419
  source 1..19: mol_type = other DNA
aaagcaacacacacatact

SEQ ID NO: 81 - DNA, 19 bp, synthetic construct
  misc_feature 1..19: note = Synthetic: V3LHS_403420
  source 1..19: mol_type = other DNA
agactgacagaaacactgg

SEQ ID NO: 82 - DNA, 19 bp, synthetic construct
  misc_feature 1..19: note = Synthetic: V3LHS_403421
  source 1..19: mol_type = other DNA
tgtctcatatattacctct

SEQ ID NO: 83 - DNA, 19 bp, synthetic construct
  misc_feature 1..19: note = Synthetic: V3LHS_403422
  source 1..19: mol_type = other DNA
tatctgaaaattattttca

SEQ ID NO: 84 - DNA, 19 bp, synthetic construct
  misc_feature 1..19: note = Synthetic: V3LHS_313522
  source 1..19: mol_type = other DNA
ttgggaagagagtaactcg

SEQ ID NO: 85 - DNA, 19 bp, synthetic construct
  misc_feature 1..19: note = Synthetic: V2LHS_206422
  source 1..19: mol_type = other DNA
tactcaatgtctttatgtg

SEQ ID NO: 86 - DNA, 19 bp, synthetic construct
  misc_feature 1..19: note = Synthetic: V3LHS_308568
  source 1..19: mol_type = other DNA
tgaatgtgatctatcagga

SEQ ID NO: 87 - DNA, 19 bp, synthetic construct
  misc_feature 1..19: note = Synthetic: V3LHS_308569
  source 1..19: mol_type = other DNA
tgttctctattatctgacg

SEQ ID NO: 88 - DNA, 19 bp, synthetic construct
  misc_feature 1..19: note = Synthetic: V3LHS_308565
  source 1..19: mol_type = other DNA
ttcatttcatatacatcca

SEQ ID NO: 89 - DNA, 19 bp, synthetic construct
  misc_feature 1..19: note = Synthetic: V3LHS_308566
  source 1..19: mol_type = other DNA
tgaacagaaagattgtgcc

SEQ ID NO: 90 - DNA, 19 bp, synthetic construct
  misc_feature 1..19: note = Synthetic: V2LHS_283849
  source 1..19: mol_type = other DNA
ataattagaggataatttg

SEQ ID NO: 91 - DNA, 19 bp, synthetic construct
  misc_feature 1..19: note = Synthetic: V3LHS_396939
  source 1..19: mol_type = other DNA
attgttgatagtgcagcct

SEQ ID NO: 92 - DNA, 19 bp, synthetic construct
  misc_feature 1..19: note = Synthetic: V3LHS_396937
  source 1..19: mol_type = other DNA
tgaatcacaagcatttccg

SEQ ID NO: 93 - DNA, 19 bp, synthetic construct
  misc_feature 1..19: note = Synthetic: V3LHS_396941
  source 1..19: mol_type = other DNA
tgatggtcatgttccggcg

SEQ ID NO: 94 - DNA, 19 bp, synthetic construct
  misc_feature 1..19: note = Synthetic: V3LHS_396940
  source 1..19: mol_type = other DNA
aataatcttgatcccagct

SEQ ID NO: 95 - DNA, 19 bp, synthetic construct
  misc_feature 1..19: note = Synthetic: V2LHS_19709
  source 1..19: mol_type = other DNA
attctgtacaattcatatg

SEQ ID NO: 96 - DNA, 19 bp, synthetic construct
  misc_feature 1..19: note = Synthetic: V2LHS_19711
  source 1..19: mol_type = other DNA
atagccagaagtaaagaac

SEQ ID NO: 97 - DNA, 19 bp, synthetic construct
  misc_feature 1..19: note = Synthetic: V2LHS_241437
  source 1..19: mol_type = other DNA
tgcggaaatatttaaggag

SEQ ID NO: 98 - DNA, 19 bp, synthetic construct
  misc_feature 1..19: note = Synthetic: V2LHS_19708
  source 1..19: mol_type = other DNA
gtaattaggagtcccacac

SEQ ID NO: 99 - DNA, 19 bp, synthetic construct
  misc_feature 1..19: note = Synthetic: V2LHS_262328
  source 1..19: mol_type = other DNA
aattaggagtcccacacag

SEQ ID NO: 100 - DNA, 19 bp, synthetic construct
  misc_feature 1..19: note = Synthetic: V3LHS_311459
  source 1..19: mol_type = other DNA
ttcttgctcagcacctcgg

SEQ ID NO: 101 - DNA, 19 bp, synthetic construct
  misc_feature 1..19: note = Synthetic: V3LHS_311462
  source 1..19: mol_type = other DNA
ttgacactgtgcagctgct

SEQ ID NO: 102 - DNA, 19 bp, synthetic construct
  misc_feature 1..19: note = Synthetic: V3LHS_311463
  source 1..19: mol_type = other DNA
taggcacaatcttgcccgc

SEQ ID NO: 103 - DNA, 19 bp, synthetic construct
  misc_feature 1..19: note = Synthetic: V2LHS_215636
  source 1..19: mol_type = other DNA
taaagcctcagaatctaag

SEQ ID NO: 104 - DNA, 19 bp, synthetic construct
  misc_feature 1..19: note = Synthetic: V2LHS_251390
  source 1..19: mol_type = other DNA
taaattacgactctgacac

SEQ ID NO: 105 - DNA, 19 bp, synthetic construct
  misc_feature 1..19: note = Synthetic: V3LHS_300082
  source 1..19: mol_type = other DNA
attatttacaacgtcaccg

SEQ ID NO: 106 - DNA, 19 bp, synthetic construct
  misc_feature 1..19: note = Synthetic: V3LHS_300078
  source 1..19: mol_type = other DNA
ttctcgtctaaaagtgcgt

SEQ ID NO: 107 - DNA, 19 bp, synthetic construct
  misc_feature 1..19: note = Synthetic: V3LHS_300081
  source 1..19: mol_type = other DNA
aaaagtgcgtggttgtccg

SEQ ID NO: 108 - DNA, 19 bp, synthetic construct
  misc_feature 1..19: note = Synthetic: V3LHS_363661
  source 1..19: mol_type = other DNA
tagctgaccgcaatcttgt

SEQ ID NO: 109 - DNA, 19 bp, synthetic construct
  misc_feature 1..19: note = Synthetic: V3LHS_363659
  source 1..19: mol_type = other DNA
tagtgaacttcttctggca

SEQ ID NO: 110 - DNA, 19 bp, synthetic construct
  misc_feature 1..19: note = Synthetic: V3LHS_363662
  source 1..19: mol_type = other DNA
tcggcttgactattggccg

SEQ ID NO: 111 - DNA, 19 bp, synthetic construct
  misc_feature 1..19: note = Synthetic: V3LHS_363664
  source 1..19: mol_type = other DNA
ttctgagactctttttccg

SEQ ID NO: 112 - DNA, 19 bp, synthetic construct
  misc_feature 1..19: note = Synthetic: V3LHS_314256
  source 1..19: mol_type = other DNA
tgtacttatccttgaaggc

SEQ ID NO: 113 - DNA, 19 bp, synthetic construct
  misc_feature 1..19: note = Synthetic: V3LHS_314257
  source 1..19: mol_type = other DNA
tgcccgcaaagtacctcca

SEQ ID NO: 114 - DNA, 19 bp, synthetic construct
  misc_feature 1..19: note = Synthetic: V2LHS_118254
  source 1..19: mol_type = other DNA
tatcccacaacttaataac

SEQ ID NO: 115 - DNA, 19 bp, synthetic construct
  misc_feature 1..19: note = Synthetic: V2LHS_118249
  source 1..19: mol_type = other DNA
taaccaaacacgaactgtc

SEQ ID NO: 116 - DNA, 19 bp, synthetic construct
  misc_feature 1..19: note = Synthetic: V3LHS_405758
  source 1..19: mol_type = other DNA
attgtatgaacaagttgga

SEQ ID NO: 117 - DNA, 19 bp, synthetic construct
  misc_feature 1..19: note = Synthetic: V3LHS_341295
  source 1..19: mol_type = other DNA
ttcacaggagtcatcttgt

SEQ ID NO: 118 - DNA, 19 bp, synthetic construct
  misc_feature 1..19: note = Synthetic: V3LHS_405756
  source 1..19: mol_type = other DNA
tatattgtatgaacaagtt

SEQ ID NO: 119 - DNA, 19 bp, synthetic construct
  misc_feature 1..19: note = Synthetic: V2LHS_243158
  source 1..19: mol_type = other DNA
atacttggcatagacactg

SEQ ID NO: 120 - DNA, 19 bp, synthetic construct
  misc_feature 1..19: note = Synthetic: V3LHS_314369
  source 1..19: mol_type = other DNA
tactgaggaatattgtgct

SEQ ID NO: 121 - DNA, 19 bp, synthetic construct
  misc_feature 1..19: note = Synthetic: V3LHS_314371
  source 1..19: mol_type = other DNA
taatgaagagactcttgcg

SEQ ID NO: 122 - DNA, 19 bp, synthetic construct
  misc_feature 1..19: note = Synthetic: V2LHS_11941
  source 1..19: mol_type = other DNA
tatgtactgacctaaatag

SEQ ID NO: 123 - DNA, 19 bp, synthetic construct
  misc_feature 1..19: note = Synthetic: V2LHS_151660
  source 1..19: mol_type = other DNA
atctgaataccaatccttc

SEQ ID NO: 124 - DNA, 19 bp, synthetic construct
  misc_feature 1..19: note = Synthetic: V3LHS_356802
  source 1..19: mol_type = other DNA
tgaacactgagcagaggtg

SEQ ID NO: 125 - DNA, 19 bp, synthetic construct
  misc_feature 1..19: note = Synthetic: V3LHS_356797
  source 1..19: mol_type = other DNA
aacagtgaacatttcacct

SEQ ID NO: 126 - DNA, 106 bp, synthetic construct
  misc_feature 1..106: note = Synthetic: l-attL
  source 1..106: mol_type = other DNA
tccgttgaagcctgcttttttatactaagttggcattataaaaaagcattgcttatcaatttgttgcaacgaacaggtcactatcagtcaaaataaaatcattatt

SEQ ID NO: 127 - DNA, 183 bp, synthetic construct
  misc_feature 1..183: note = Synthetic: l-attR
  source 1..183: mol_type = other DNA
agatgcctcagctctgttacaggtcactaataccatctaagtagttgattcatagtgactgcatatgttgtgttttacagtattatgtagtctgttttttatgcaaaatctaatttaatatattgatatttatatcattttacgtttctcgttcagcttttttatactaacttgagcgaaacg

SEQ ID NO: 128 - DNA, 41 bp, synthetic construct
  misc_feature 1..41: note = Synthetic: l-attB
  source 1..41: mol_type = other DNA
tccgttgaagcctgcttttttatactaacttgagcgaaacg

SEQ ID NO: 129 - DNA, 248 bp, synthetic construct
  misc_feature 1..248: note = Synthetic: l-attP
  source 1..248: mol_type = other DNA
agatgcctcagctctgttacaggtcactaataccatctaagtagttgattcatagtgactgcatatgttgtgttttacagtattatgtagtctgttttttatgcaaaatctaatttaatatattgatatttatatcattttacgtttctcgttcagcttttttatactaagttggcattataaaaaagcattgcttatcaatttgttgcaacgaacaggtcactatcagtcaaaataaaatcattatt

SEQ ID NO: 130 - DNA, 34 bp, synthetic construct
  misc_feature 1..34: note = Synthetic: loxP
  source 1..34: mol_type = other DNA
ataacttcgtatagcatacattatacgaagttat

SEQ ID NO: 131 - DNA, 130 bp, synthetic construct
  misc_feature 1..130: note = Synthetic: gd-res
  source 1..130: mol_type = other DNA
attttgcaaccgtccgaaatattataaattatcgcacacataaaaacagtgctgttaatgtgtctattaaatcgattttttgttataacagacactgcttgtccgatatttgatttaggatacattttta

SEQ ID NO: 132 - DNA, 34 bp, synthetic construct
  misc_feature 1..34: note = Synthetic: FRT
  source 1..34: mol_type = other DNA
gaagttcctattctctagaaagtataggaacttc

SEQ ID NO: 133 - DNA, 26 bp, synthetic construct
  misc_feature 1..26: note = Synthetic: hixL
  source 1..26: mol_type = other DNA
ttcttgaaaaccaaggtttttgataa

SEQ ID NO: 134 - DNA, 26 bp, synthetic construct
  misc_feature 1..26: note = Synthetic: hixR
  source 1..26: mol_type = other DNA
ttttccttttggaaggtttttgataa

SEQ ID NO: 135 - DNA, 121 bp, synthetic construct
  misc_feature 1..121: note = Synthetic: Tn3 res
  source 1..121: mol_type = other DNA
caaccgttcgaaatattataaattatcagacatagtaaaacggcttcgtttgagtgtccattaaatcgtcattttggcataatagacacatcgtgtctgatattcgatttaaggtacattt

SEQ ID NO: 136 - DNA, 126 bp, synthetic construct
  misc_feature 1..126: note = Synthetic: Tn21 res
  source 1..126: mol_type = other DNA
gccgccgtcaggttgaggcataccctaacctgatgtcagatgccatgtgtaaattgcgtcaggataggattgaattttgaatttattgacatatctcgttgaaggtcatagagtcttccctgacat

SEQ ID NO: 137 - DNA, 30 bp, synthetic construct
  misc_feature 1..30: note = Synthetic: cer
  source 1..30: mol_type = other DNA
ggtgcgtacaattaagggattatggtaaat

SEQ ID NO: 138 - DNA, 28 bp, synthetic construct
  misc_feature 1..28: note = Synthetic: psi
  source 1..28: mol_type = other DNA
ggtgcgcgcaagatccattatgttaaac

SEQ ID NO: 139 - DNA, 584 bp, unidentified
  misc_feature 1..584: note = Promoter from the human cytomegalovirus (CMV)
  source 1..584: mol_type = unassigned DNA
gacattgattattgactagttattaatagtaatcaattacggggtcattagttcatagcccatatatggagttccgcgttacataacttacggtaaatggcccgcctggctgaccgcccaacgacccccgcccattgacgtcaataatgacgtatgttcccatagtaacgccaatagggactttccattgacgtcaatgggtggagtatttacggtaaactgcccacttggcagtacatcaagtgtatcatatgccaagtacgccccctattgacgtcaatgacggtaaatggcccgcctggcattatgcccagtacatgaccttatgggactttcctacttggcagtacatctacgtattagtcatcgctattaccatggtgatgcggttttggcagtacatcaatgggcgtggatagcggtttgactcacggggatttccaagtctccaccccattgacgtcaatgggagtttgttttggcaccaaaatcaacgggactttccaaaatgtcgtaacaactccgccccattgacgcaaatgggcggtaggcgtgtacggtgggaggtctatataagcagagct

SEQ ID NO: 140 - DNA, 100 bp, unidentified
  misc_feature 1..100: note = mini-CMV
  source 1..100: mol_type = unassigned DNA
ccaaaatcaacgggactttccaaaatgtcgtaacaactccgccccattgacgcaaatgggcggtaggcgtgtacggtgggaggtctatataagcagagct

SEQ ID NO: 141 - DNA, 262 bp, Rous sarcoma virus
  misc_feature 1..262: note = Long terminal repeat (LTR) of the rous sarcoma virus (RSV)
  source 1..262: mol_type = genomic DNA
ggtgcacaccaatgtggtgaatggtcaaatggcgtttattgtatcgagctaggcacttaaatacaatatctctgcaatgcggaattcagtggttcgtccaatccatgtcagacccgtctgttgccttcctaataaggcacgatcgtaccaccttacttccaccaatcggcatgcacggtgctttttctctccttgtaaggcatgttgctaactcatcgttaccatgttgcaagactacaagagtattgcataagactacatt

SEQ ID NO: 142 - DNA, 584 bp, synthetic construct
  misc_feature 1..584: note = Synthetic: CAG
  source 1..584: mol_type = other DNA
gcgttacataacttacggtaaatggcccgcctggctgaccgcccaacgacccccgcccattgacgtcaataatgacgtatgttcccatagtaacgccaatagggactttccattgacgtcaatgggtggagtatttacggtaaactgcccacttggcagtacatcaagtgtatcatatgccaagtacgccccctattgacgtcaatgacggtaaatggcccgcctggcattatgcccagtacatgaccttatgggactttcctacttggcagtacatctacgtattagtcatcgctattaccatggtcgaggtgagccccacgttctgcttcactctccccatctcccccccctccccacccccaattttgtatttatttattttttaattattttgtgcagcgatgggggcggggggggggggggggcgcgcgccaggcggggcggggcggggcgaggggcggggcggggcgaggcggagaggtgcggcggcagccaatcagagcggcgcgctccgaaagtttccttttatggcgaggcggcggcggcggcggccctataaaaagcgaagcgcgcggcgggcg

SEQ ID NO: 143 - DNA, 1182 bp, Homo sapiens
  misc_feature 1..1182: note = EF1a
  source 1..1182: mol_type = genomic DNA
gctccggtgcccgtcagtgggcagagcgcacatcgcccacagtccccgagaagttggggggaggggtcggcaattgaaccggtgcctagagaaggtggcgcggggtaaactgggaaagtgatgtcgtgtactggctccgcctttttcccgagggtgggggagaaccgtatataagtgcagtagtcgccgtgaacgttctttttcgcaacgggtttgccgccagaacacaggtaagtgccgtgtgtggttcccgcgggcctggcctctttacgggttatggcccttgcgtgccttgaattacttccacgcccctggctgcagtacgtgattcttgatcccgagcttcgggttggaagtgggtgggagagttcgaggccttgcgcttaaggagccccttcgcctcgtgcttgagttgaggcctggcctgggcgctggggccgccgcgtgcgaatctggtggcaccttcgcgcctgtctcgctgctttcgataagtctctagccatttaaaatttttgatgacctgctgcgacgctttttttctggcaagatagtcttgtaaatgcgggccaagatctgcacactggtatttcggtttttggggccgcgggcggcgacggggcccgtgcgtcccagcgcacatgttcggcgaggcggggcctgcgagcgcggccaccgagaatcggacgggggtagtctcaagctggccggcctgctctggtgcctggcctcgcgccgccgtgtatcgccccgccctgggcggcaaggctggcccggtcggcaccagttgcgtgagcggaaagatggccgcttcccggccctgctgcagggagctcaaaatggaggacgcggcgctcgggagagcgggcgggtgagtcacccacacaaaggaaaagggcctttccgtcctcagccgtcgcttcatgtgactccacggagtaccgggcgccgtccaggcacctcgattagttctcgagcttttggagtacgtcgtctttaggttggggggaggggttttatgcgatggagtttccccacactgagtgggtggagactgaagttaggccagcttggcacttgatgtaattctccttggaatttgccctttttgagtttggatcttggttcattctcaagcctcagacagtggttcaaagtttttttcttccatttcaggtgtcgtga

SEQ ID NO: 144 - DNA, 251 bp, synthetic construct
  misc_feature 1..251: note = Synthetic: EFS
  source 1..251: mol_type = other DNA
atcgattggctccggtgcccgtcagtgggcagagcgcacatcgcccacagtccccgagaagttggggggaggggtcggcaattgaaccggtgcctagagaaggtggcgcggggtaaactgggaaagtgatgtcgtgtactggctccgcctttttcccgagggtgggggagaaccgtatataagtgcagtagtcgccgtgaacgttctttttcgcaacgggtttgccgccagaacacaggtgtcgtgacgcg

SEQ ID NO: 145 - DNA, 1212 bp, Homo sapiens
  misc_feature 1..1212: note = Human b-actin
  source 1..1212: mol_type = genomic DNA
ggcctccgcgccgggttttggcgcctcccgcgggcgcccccctcctcacggcgagcgctgccacgtcagacgaagggcgcagcgagcgtcctgatccttccgcccggacgctcaggacagcggcccgctgctcataagactcggccttagaaccccagtatcagcagaaggacattttaggacgggacttgggtgactctagggcactggttttctttccagagagcggaacaggcgaggaaaagtagtcccttctcggcgattctgcggagggatctccgtggggcggtgaacgccgatgattatataaggacgcgccgggtgtggcacagctagttccgtcgcagccgggatttgggtcgcggttcttgtttgtggatcgctgtgatcgtcacttggtgagtagcgggctgctgggctggccggggctttcgtggccgccgggccgctcggtgggacggaagcgtgtggagagaccgccaagggctgtagtctgggtccgcgagcaaggttgccctgaactgggggttggggggagcgcagcaaaatggcggctgttcccgagtcttgaatggaagacgcttgtgaggcgggctgtgaggtcgttgaaacaaggtggggggcatggtgggcggcaagaacccaaggtcttgaggccttcgctaatgcgggaaagctcttattcgggtgagatgggctggggcaccatctggggaccctgacgtgaagtttgtcactgactggagaactcggtttgtcgtctgttgcgggggcggcagttatggcggtgccgttgggcagtgcacccgtacctttgggagcgcgcgccctcgtcgtgtcgtgacgtcacccgttctgttggcttataatgcagggtggggccacctgccggtaggtgtgcggtaggcttttctccgtcgcaggacgcagggttcgggcctagggtaggctctcctgaatcgacaggcgccggacctctggtgaggggagggataagtgaggcgtcagtttctttggtcggttttatgtacctatcttcttaagtagctgaagctccggttttgaactatgcgctcggggttggcgagtgtgttttgtgaagttttttaggcaccttttgaaatgtaatcatttgggtcaatatgtaattttcagtgttagactagtaaattgtccgctaaattctggccgtttttggcttttttgttagac

SEQ ID NO: 146 - DNA, 211 bp, unidentified
  misc_feature 1..211: note = NFK-b
  source 1..211: mol_type = unassigned DNA
gctagcgggaatttccgggaatttccgggaatttccgggaatttccagatctgccgccccgactgcatctgcgtgttcgaattcgccaatgacaagacgctgggcggggtttgtgtcatcatagaactaaagacatgcaaatatatttcttccggggacaccgccagcaaacgcgagcaacgggccacggggatgaagcagaagcttggca

SEQ ID NO: 147 - DNA, 1211 bp, Homo sapiens
  misc_feature 1..1211: note = Ubiquitin-C
  source 1..1211: mol_type = genomic DNA
gtctaacaaaaaagccaaaaacggccagaatttagcggacaatttactagtctaacactgaaaattacatattgacccaaatgattacatttcaaaaggtgcctaaaaaacttcacaaaacacactcgccaaccccgagcgcatagttcaaaaccggagcttcagctacttaagaagataggtacataaaaccgaccaaagaaactgacgcctcacttatccctcccctcaccagaggtccggcgcctgtcgattcaggagagcctaccctaggcccgaaccctgcgtcctgcgacggagaaaagcctaccgcacacctaccggcaggtggccccaccctgcattataagccaacagaacgggtgacgtcacgacacgacgagggcgcgcgctcccaaaggtacgggtgcactgcccaacggcaccgccataactgccgcccccgcaacagacgacaaaccgagttctccagtcagtgacaaacttcacgtcagggtccccagatggtgccccagcccatctcacccgaataagagctttcccgcattagcgaaggcctcaagaccttgggttcttgccgcccaccatgccccccaccttgtttcaacgacctcacagcccgcctcacaagcgtcttccattcaagactcgggaacagccgccattttgctgcgctccccccaacccccagttcagggcaaccttgctcgcggacccagactacagcccttggcggtctctccacacgcttccgtcccaccgagcggcccggcggccacgaaagccccggccagcccagcagcccgctactcaccaagtgacgatcacagcgatccacaaacaagaaccgcgacccaaatcccggctgcgacggaactagctgtgccacacccggcgcgtccttatataatcatcggcgttcaccgccccacggagatccctccgcagaatcgccgagaagggactacttttcctcgcctgttccgctctctggaaagaaaaccagtgccctagagtcacccaagtcccgtcctaaaatgtccttctgctgatactggggttctaaggccgagtcttatgagcagcgggccgctgtcctgagcgtccgggcggaaggatcaggacgctcgctgcgcccttcgtctgacgtggcagcgctcgccgtgaggaggggggcgcccgcgggaggcgccaaaacccggcgcggaggc

SEQ ID NO: 148 - DNA, 317 bp, unidentified
  misc_feature 1..317: note = SV40
  source 1..317: mol_type = unassigned DNA
ggtgtggaaagtccccaggctccccagcaggcagaagtatgcaaagcatgcatctcaattagtcagcaaccaggtgtggaaagtccccaggctccccagcaggcagaagtatgcaaagcatgcatctcaattagtcagcaaccatagtcccgcccctaactccgcccatcccgcccctaactccgcccagttccgcccattctccgccccatggctgactaattttttttatttatgcagaggccgaggccgcctcggcctctgagctattccagaagtagtgaggaggcttttttggaggcctaggcttttgcaaa

SEQ ID NO: 149 - DNA, 399 bp, unidentified
  misc_feature 1..399: note = PGK
  source 1..399: mol_type = unassigned DNA
ccggtaggcgccaaccggctccgttctttggtggccccttcgcgccaccttctactcctcccctagtcaggaagttcccccccgccccgcagctcgcgtcgtgcaggacgtgacaaatggaagtagcacgtctcactagtctcgtgcagatggacagcaccgctgagcaatggaagcgggtaggcctttggggcagcggccaatagcagctttgctccttcgctttctgggctcagaggctgggaaggggtgggtccgggggcgggctcaggggcgggctcaggggcggggcgggcgcccgaaggtcctccggaggcccggcattctgcacgcttcaaaagcgcacgtctgccgcgctgttctcctcttcctcatctccgggcctttcgacctgcagcc

SEQ ID NO: 150 - DNA, 99 bp, synthetic construct
  misc_feature 1..99: note = Synthetic: H1
  source 1..99: mol_type = other DNA
aatatttgcatgtcgctatgtgttctgggaaatcaccataaacgtgaaatgtctttggatttgggaatcttataagttctgtatgagaccacagatccc

SEQ ID NO: 151 - DNA, 314 bp, Homo sapiens
  misc_feature 1..314: note = U6
  source 1..314: mol_type = genomic DNA
gatccgacgccgccatctctaggcccgcgccggccccctcgcacagacttgtgggagaagctcggctactcccctgccccggttaatttgcatataatatttcctagtaactatagaggcttaatgtgcgataaaagacagataatctgttctttttaatactagctacattttacatgataggcttggatttctataagagatacaaatactaaattattattttaaaaaacagcacaaaaggaaactcaccctaactgtaaagtaattgtgtgttttgagactataaatatcccttggagaaaagccttgtt

SEQ ID NO: 152 - DNA, 250 bp, synthetic construct
  misc_feature 1..250: note = Synthetic: 250 bp S/MAR
  source 1..250: mol_type = other DNA
tctttaatttctaatatatttagaatctttaatttctaatatatttagaatctttaatttctaatatatttagaatctttaatttctaatatatttagaatctttaatttctaatatatttagaatctttaatttctaatatatttagaatctttaatttctaatatatttagaatctttaatttctaatatatttagaatctttaatttctaatatatttagaatctttaatttctaatatatttagaa

SEQ ID NO: 153 - DNA, 250 bp, synthetic construct; identical to SEQ ID NO: 152
  misc_feature 1..250: note = Synthetic: 439 bp S/MAR
  source 1..250: mol_type = other DNA

SEQ ID NO: 154 - DNA, 45 bp, synthetic construct
  misc_feature 1..45: note = Synthetic: (45 bp) Type A
  source 1..45: mol_type = other DNA
ggtgcatcgatgcagcatcgaggcaggtgcatcgatacagggggg

SEQ ID NO: 155 - DNA, 24 bp, synthetic construct
  misc_feature 1..24: note = Synthetic: (24 bp) Type B
  source 1..24: mol_type = other DNA
tcgtcgttttgtcgttttgtcgtt

SEQ ID NO: 156 - DNA, 21 bp, synthetic construct
  misc_feature 1..21: note = Synthetic: (21 bp) Type C
  source 1..21: mol_type = other DNA
tcgtcgaacgttcgagatgat

SEQ ID NO: 157 - DNA, 130 bp, synthetic construct
  misc_feature 1..130: note = Synthetic: Beta-globin intron
  source 1..130: mol_type = other DNA
gttggtatcaaggttacaagacaggtttaaggagaccaatagaaactgggcatgtggagacagagaagactcttgggtttctgataggcactgactctctctgcctattggtctattttcccacccttag

SEQ ID NO: 158 - DNA, 262 bp, Homo sapiens
  misc_feature 1..262: note = Human growth hormone intron
  source 1..262: mol_type = genomic DNA
ttcgaacaggtaagcgcccctaaaatccctttgggcacaatgtgtcctgaggggagaggcagcgacctgtagatgggacgggggcactaaccctcaggtttggggcttctgaatgtgagtatcgccatgtaagcccagtatttggccaatctcagaaagctcctggtccctggagggatggagagagaaaaacaaacagctcctggagcagggagagtgctggcctcttgctctccggctccctctgttgccctctggtttc

SEQ ID NO: 159 - DNA, 55 bp, unidentified
  misc_feature 1..55: note = NF-kb
  source 1..55: mol_type = unassigned DNA
ggggactttccggggactttccggggactttccggggactttccggggactttcc

SEQ ID NO: 160 - DNA, 20 bp, unidentified
  misc_feature 1..20: note = p53 NLS
  source 1..20: mol_type = unassigned DNA
agactgggcatgtctgggca

SEQ ID NO: 161 - DNA, 20 bp, unidentified
  misc_feature 1..20: note = p53 NLS
  source 1..20: mol_type = unassigned DNA
gaacatgtcccaacatgttg

SEQ ID NO: 162 - DNA, 15 bp, unidentified
  misc_feature 1..15: note = Adeno-virus major late promoter
  source 1..15: mol_type = unassigned DNA
ggggctataaaaggg